European Patent Specification EP 3 515 475 B1, published May 1, 2024. Title: CHIMERIC ANTIGEN RECEPTOR (CAR) THAT TARGETS CHEMOKINE RECEPTOR CCR4 AND ITS USE. Applicant: THE UNITED STATES OF AMERICA, as represented by the Secretary, Department of Health and Human Services Perera, Liyanage P Waldmann, Thomas. The sequence listing filed with the application follows.

SEQUENCE LISTING (19 sequences)

SEQ ID NO: 1 - protein, 118 aa, Artificial Sequence
  VH of humanized affinity matured mAb1567
QVQLVQSGAEVKKPGASVKVSCKASGYTFASAWMHWMRQAPGQGLEWIGWINPGNVNTKYNEKFKGRATLTVDTSTNTAYMELSSLRSEDTAVYYCARSTYYRPLDYWGQGTLVTVSS

SEQ ID NO: 2 - protein, 112 aa, Artificial Sequence
  VL of humanized affinity matured mAb1567
DIVMTQSPDSLAVSLGERATINCKSSQSILYSSNQKNYLAWYQQKPGQSPKLLIYWASTRESGVPDRFSGSGSGTDFTLTISSLQAEDVAVYYCHQYMSSYTFGQGTKLEIK

SEQ ID NO: 3 - protein, 17 aa, Artificial Sequence
  Linker
SSGGGGSGGGGSGGGGS

SEQ ID NO: 4 - protein, 22 aa, Artificial Sequence
  Signal protein
MDFQVQIFSFLLISASVIMSRG

SEQ ID NO: 5 - protein, 22 aa, Artificial Sequence
  Signal Protein
LLVTSLLLCELPHPAFLLIPDT

SEQ ID NO: 6 - protein, 236 aa, Artificial Sequence
  Immunoglobulin Domain
EPKSCDKTHTCPPCPAPELLGGPSVFLFPPKPKDTLMISRTPEVTCVVVDVSHEDPEVKFNWYVDGVEVHNAKTKPREEQYNSTYRVVSVLTVLHQDWLNGKEYKCKVSNKALPAPIEKTISKAKGQPREPQVYTLPPSRDELTKNQVSLTCLVKGFYPSDIAVEWESNGQPENNYKTTPPVLDSDGSFFLYSKLTVDKSRWQQGNVFSCSVMHEALHNHYTQKSLSLSPGKKDPK

SEQ ID NO: 7 - protein, 93 aa, Artificial Sequence
  CD8 Transmembrane Domain
ALSNSIMYFSHFVPVFLPAKPTTTPAPRPPTPAPTIASQPLSLRPEACRPAAGGAVHTRGLDFACDIYIWAPLAGTCGVLLLSLVITLYCNHR

SEQ ID NO: 8 - protein, 42 aa, Artificial Sequence
  4-1BB Signalling Domain
KRGRKKLLYIFKQPFMRPVQTTQEEDGCSCRFPEEEEGGCEL

SEQ ID NO: 9 - protein, 112 aa, Artificial Sequence
  CD3 zeta domain
RVKFSRSADAPAYQQGQNQLYNELNLGRREEYDVLDKRRGRDPEMGGKPRRKNPQEGLYNELQKDKMAEAYSEIGMKGERRRGKGHDGLYQGLSTATKDTYDALHMQALPPR

SEQ ID NO: 10 - protein, 516 aa, Artificial Sequence
  Chimeric Antigen Receptor
MDFQVQIFSFLLISASVIMSRGDIVMTQSPDSLAVSLGERATINCKSSQSILYSSNQKNYLAWYQQKPGQSPKLLIYWASTRESGVPDRFSGSGSGTDFTLTISSLQAEDVAVYYCHQYMSSYTFGQGTKLEIKSSGGGGSGGGGSGGGGSQVQLVQSGAEVKKPGASVKVSCKASGYTFASAWMHWMRQAPGQGLEWIGWINPGNVNTKYNEKFKGRATLTVDTSTNTAYMELSSLRSEDTAVYYCARSTYYRPLDYWGQGTLVTVSSALSNSIMYFSHFVPVFLPAKPTTTPAPRPPTPAPTIASQPLSLRPEACRPAAGGAVHTRGLDFACDIYIWAPLAGTCGVLLLSLVITLYCNHRKRGRKKLLYIFKQPFMRPVQTTQEEDGCSCRFPEEEEGGCELRVKFSRSADAPAYQQGQNQLYNELNLGRREEYDVLDKRRGRDPEMGGKPRRKNPQEGLYNELQKDKMAEAYSEIGMKGERRRGKGHDGLYQGLSTATKDTYDALHMQALPPR

SEQ ID NO: 11 - DNA, 66 bp, Artificial Sequence
  DNA encoding signal sequence
atggactttcaagtgcagatctttagtttcctgctcataagcgctagtgtgatcatgtccagagga

SEQ ID NO: 12 - DNA, 336 bp, Artificial Sequence
  DNA encoding VL of humanized affinity matured  mAb1567
gatattgtgatgactcaaagccccgacagtctggccgtgtctttgggcgagagagccacaatcaactgcaagtcctcacagagtatcctttattcctctaatcagaagaattacctcgcatggtatcaacaaaaacccggacagagccctaagcttttgatctattgggcatctacccgagaatcaggagtgccggaccgcttcagtggatcaggatcaggcacagactttacgctgacaatatcctctcttcaggccgaagacgttgccgtgtactactgccatcaatatatgtcaagctacacattcggccagggcaccaaactcgagattaag

SEQ ID NO: 13 - DNA, 354 bp, Artificial Sequence
  DNA encoding VH of humanized affinity matured  mAb1567
caggttcagctcgtgcaatcaggggcagaggtcaagaagccgggtgcctctgtgaaggtgtcatgtaaggcctccgggtatacttttgccagcgcctggatgcattggatgaggcaggcgcccggccagggtctggagtggattggttggattaatcccggaaacgtgaatactaagtataacgagaagtttaagggcagggccacactcacagtcgacacaagcaccaataccgcgtacatggaactttccagcctccggtccgaggacactgcggtgtattactgcgcacgctccacctattacagaccacttgattactggggccaagggaccctggtgaccgtgtctagc

SEQ ID NO: 14 - DNA, 51 bp, Artificial Sequence
  DNA encoding a linker
tctagtggtggcggaggcagtggcggaggaggctccgggggcggagggtcc

SEQ ID NO: 15 - DNA, 279 bp, Artificial Sequence
  DNA encoding CD8 domains
gcactcagcaattccatcatgtacttctctcatttcgtgccagtatttctgcctgccaagccaactaccacacctgcgccacgccctcccacgcccgcacccacaattgcttcacagcctctttctctgcggcctgaggcttgtcgcccagcagccggaggcgccgtgcatacgcgcggccttgacttcgcatgtgacatctacatttgggctcctttggctggaacctgcggggtgttgttgcttagtctggtgattaccctctactgcaatcataga

SEQ ID NO: 16 - DNA, 126 bp, Artificial Sequence
  DNA encoding 4-1BB signaling molecule
aagcgggggcgaaagaaacttctctatatcttcaaacagcctttcatgcgaccagtgcagacaacccaagaggaagacggatgcagctgtcgctttccagaggaggaagaagggggctgcgagctg

SEQ ID NO: 17 - DNA, 306 bp, Artificial Sequence
  DNA encoding a CD3 zeta domain
agagtgaaattctctcgctccgctgacgcccccgcgtatcaacagggccagaatcagctctacaacgaacttaaccttgggcggagagaagaatacgatgttctcgacaagcgcagggggagagaccctgagatgggcgggaaaccgcgccgcaagaacccccaagaagggttgtataacgagctccagaaggacaaaatggctgaagcctactcagagataggtatgaagggcgagcgccgcagagggaagggacacgatggtctgtaccaaggcctttcaaccgccaccaaggatacctatgat

SEQ ID NO: 18 - DNA, 1565 bp, Artificial Sequence
  DNA encoding a chimeric antigen receptor
gcggccgcatggactttcaagtgcagatctttagtttcctgctcataagcgctagtgtgatcatgtccagaggagatattgtgatgactcaaagccccgacagtctggccgtgtctttgggcgagagagccacaatcaactgcaagtcctcacagagtatcctttattcctctaatcagaagaattacctcgcatggtatcaacaaaaacccggacagagccctaagcttttgatctattgggcatctacccgagaatcaggagtgccggaccgcttcagtggatcaggatcaggcacagactttacgctgacaatatcctctcttcaggccgaagacgttgccgtgtactactgccatcaatatatgtcaagctacacattcggccagggcaccaaactcgagattaagtctagtggtggcggaggcagtggcggaggaggctccgggggcggagggtcccaggttcagctcgtgcaatcaggggcagaggtcaagaagccgggtgcctctgtgaaggtgtcatgtaaggcctccgggtatacttttgccagcgcctggatgcattggatgaggcaggcgcccggccagggtctggagtggattggttggattaatcccggaaacgtgaatactaagtataacgagaagtttaagggcagggccacactcacagtcgacacaagcaccaataccgcgtacatggaactttccagcctccggtccgaggacactgcggtgtattactgcgcacgctccacctattacagaccacttgattactggggccaagggaccctggtgaccgtgtctagcgcactcagcaattccatcatgtacttctctcatttcgtgccagtatttctgcctgccaagccaactaccacacctgcgccacgccctcccacgcccgcacccacaattgcttcacagcctctttctctgcggcctgaggcttgtcgcccagcagccggaggcgccgtgcatacgcgcggccttgacttcgcatgtgacatctacatttgggctcctttggctggaacctgcggggtgttgttgcttagtctggtgattaccctctactgcaatcatagaaagcgggggcgaaagaaacttctctatatcttcaaacagcctttcatgcgaccagtgcagacaacccaagaggaagacggatgcagctgtcgctttccagaggaggaagaagggggctgcgagctgagagtgaaattctctcgctccgctgacgcccccgcgtatcaacagggccagaatcagctctacaacgaacttaaccttgggcggagagaagaatacgatgttctcgacaagcgcagggggagagaccctgagatgggcgggaaaccgcgccgcaagaacccccaagaagggttgtataacgagctccagaaggacaaaatggctgaagcctactcagagataggtatgaagggcgagcgccgcagagggaagggacacgatggtctgtaccaaggcctttcaaccgccaccaaggatacctatgatgcactgcacatgcaagccctgcctcctcgctaaggatcc

SEQ ID NO: 19 - protein, 67 aa, Artificial Sequence
  CD28 transmembrane domain
IEVMYPPPYLDNEKSNGTIIHVKGKHLCPSPLFPGPSKPFWVLVVVGGVLACYSLLVTVAFIIFWVR